European Patent Application EP 4 129 293 A1, published February 8, 2023. Title: Neuronal degeneration inhibitor. Applicant: Kyoto University TAKEDA PHARMACEUTICAL COMPANY LIMITED. The sequence listing filed with the application follows.

SEQUENCE LISTING (1 sequence)

SEQ ID NO: 1 - DNA, 24 bp, Artificial Sequence
  DNA probe
ccccggccccggccccggccccgg